European Patent Specification EP 4 532 758 B1, published July 1, 2026. Title: Adaptor ligation. Applicant: Epigenica AB. Application EP 22175502.8, filed May 25, 2022. The sequence listing filed with the application follows.

SEQUENCE LISTING (126 sequences)

SEQ ID NO: 1 - protein, 198 aa, Escherichia coli
MIEFVYPHTHLVAGVDEVGRGPLVGAVVTAAVILDPARPIAELNDSKKLSEKRRLALCEEIKEKALSWSLGRAEPYEIDELNILHATMLAMQRAVAGLHIAPEYVLIDGNRCPKLPMPSMAVVKGDSRVPEISAASILAKVTRDAEMAALDIVFPQYGFAQHKGYPTAFHLEKLAEYGATEHHRRSFGPVKRALGLAS

SEQ ID NO: 2 - protein, 198 aa, Salmonella bongori
MIEFVYPHTHLVAGVDEVGRGPLVGAVVTAAVILDPARPIVGLNDSKKLSEKRRLALYDEIKEKALSWSLGRAEPHEIDELNILHATMLAMQRAVAGLHIAPEYVLIDGNRCPALPVPSMAVVKGDSRVAEISAASILAKVTRDAEMAALDIVFPQYGFAQHKGYPTAFHLEKLAQYGATAHHRRSFAPVKRALGLAS

SEQ ID NO: 3 - protein, 198 aa, Enterobacter lignolyticus
MMEFIYPHTHLVAGVDEVGRGPLVGAVVTAAVILDPARPIVGLNDSKKLSEKRRLALFDEIKEKALCWSLGRAEPHEIDELNILHATMLAMQRAVAGLHITPEYVLIDGNRCPALPVPSMAVVKGDSRVAEISAASILAKVTRDAEMAELDVTFPQYGFAQHKGYPTAFHLEKLAEHGPTEHHRRSFGPVKRALGLAS

SEQ ID NO: 4 - protein, 194 aa, Cronobacter sakazakii
MMEFIYPHTHLVAGVDEVGRGPLVTAAVILDPLKPIVGLADSKKLSEKRRLALFDEIKEKAIAWSLGRAEPHEIDELNILHATMLAMQRAVAGLAVTPEYVLVDGNRCPALPMPSMAVVKGDSRVAEISAASILAKVTRDAEMAELDLTFPQYGFAQHKGYPTAFHLERLAEHGATAHHRRSFAPVRRALGIAS

SEQ ID NO: 5 - protein, 198 aa, Jejubacter calystegiae
MMEFVYPHTRLVAGVDEVGRGPLVGAVVTAAVILDPERPIAGLADSKKLSEKRRQALHDEICEKALAWSLGRAEPHEIDQLNILHATMLAMQRAVAGLAIAPEYVLIDGNRCPTLPVPSMAVIKGDGLVAEISAASIIAKVSRDREMAELDRAFPEYGFAKHKGYPTALHLEKLAQYGATEHHRRSFAPVKRALGLSA

SEQ ID NO: 6 - protein, 198 aa, Yersinia aldovae
MNDIFIYPQANLIAGVDEVGRGPLVGAVVTAAVILDPKRPIVGLADSKKLSEKRRLSLYDEITDKALSWSLGRAEPEEIDQLNILHATMLAMQRAVAGLHIAPDYVLIDGNRCPKLAMPSLAVVKGDSRVAEISAASILAKVTRDGEMTELDLSFPGYGFAQHKGYPTAFHLERLAALGATEHHRRSFGPVKRVLGLV

SEQ ID NO: 7 - protein, 197 aa, Mangrovibacter phragmitis
MSEFIYPHTYRVAGVDEVGRGPLVGAVVTAAVILDPARPISGLADSKKLSEKRRLSLYDEIVDKALAWSLGRAEPAEIDSLNILHATMLAMQRAVAGLSISPEYVLIDGNRCPVLPVPSMAVVKGDSLVAEISAASILAKVTRDKEMVELDLQYPEYGFAQHKGYPTAYHLEKLAALGATEHHRRSFSPVKRALGLA

SEQ ID NO: 8 - protein, 198 aa, Serratia sp. ATCC 39006
MNKSFSYPQATCIAGVDEVGRGPLVGAVVTAAVILDPNRPIVGLADSKKLSEKRRLSLYDEIKDKALAWSLGRAEPEEIDQLNILHATMLAMQRAVAGLVLTPDYVLIDGNRCPMLPMPSLAVVKGDDLVPEISAASILAKVTRDWEMEALDKIFPAYGFAQHKGYPTAYHLEKLATLGATHHHRSSFAPVKRALGLA

SEQ ID NO: 9 - protein, 198 aa, Pectobacterium punjabense
MSEIFIYPQANCIAGVDEVGRGPLVGAVVTAAVILDPTRPIVGLADSKKLSEKRRLALYDEIKEKALAWSLGRAEPEEIDQLNILHATMLAMQRAVAGLSIVPDFVLIDGNRSPALSMPAQAVVKGDSRVAEISAASIMAKVTRDREMVELDQRFPAYGFAQHKGYPTAFHLEKLAALGATEFHRRSFAPVKRALGLA

SEQ ID NO: 10 - protein, 196 aa, Photorhabdus sp. UCH-936
MMEFIYPQASLIAGVDEVGRGPLVGAVVTAAVILDPSRPITGLADSKKLSEKRREALYLEITEKALCWSLGRAEPEEIDQLNILHATMLAMQRAVAGLSIPPEYVLIDGNRCPKLSIPAQAVIKGDGLVAEISAASIVAKVTRDREMAELDQLFPEYGFAKHKGYPTAFHLEKLALLGATKHHRKSFAPVKRAIGL

SEQ ID NO: 11 - protein, 197 aa, Edwardsiella
MSEIFVYPCADRIAGVDEVGRGPLVGAVVTAAVILDPARPIAGLADSKKLSEKRRCALYDEIVEKALCWSLGRAEAEEIDRLNILQATMVAMQRAVAGLALQPDFVLIDGNRCPALPMAAQAVVKGDSRVAEISAASILAKVTRDREMAELDCCYPEYGFAQHKGYPTALHLERLAALGATEHHRRSFGPVKRVLGL

SEQ ID NO: 12 - protein, 208 aa, Pantoea allii
MADFIYPAARCIAGVDEVGRGPLVGAVVTAAVILDPANPIPGLADSKKLSEKRRLALFDQIKEKALAWSLGRAEPEEIDRLNILHATMLAMQRAVAGLPLTPDFVLIDGNRCPALPMPSLAVVKGDSLVAEISAASIIAKVTRDREMAELDLLFPQYGFAQHKGYPTALHREKLTQYGATPHHRRSFAPVRNALIDADVLASSLTTLR

SEQ ID NO: 13 - protein, 205 aa, Klebsiella michiganensis
MMEFVYPHTHLVAGVDEVGRGPLVGAVVTAAVILDPAKPIVGLNDSKKLSEKRRLALFDEIKEKALCWSLGRAEPHEIDELNILHATMLAMQRAVAGLRVSPEFVLIDGNRCPPLPMPSLAVVKGDSRVAEISAASILAKVTRDAEMAVLDREFPQYGFAQHKGYPTAFHLQKAAGTWRNRAIPAQLWPGETRAGPGVLNRHASN

SEQ ID NO: 14 - protein, 197 aa, Ewingella americana
MSDIFVYPQALCIAGVDEVGRGPLVGAVVTAAVILDPAKPILGLADSKKLTEKRREALYIEIKEKALSWSLGRAEPDEIDELNILHATMLAMQRAVAGLHITPDMVLIDGNRCPKLPMASQAVVKGDSKVAEISAASILAKVTRDREMVELDLQFPDYGFAKHKGYPTPVHLESLAKLGATPHHRRSFAPVRRALGQ

SEQ ID NO: 15 - protein, 198 aa, Biostraticola tofi
MTELFVYPPATSIAGVDEVGRGPLVGAVVTAAVILDPKRPIIGLADSKKLSEKRRLSLYDEITDKALAWSLGRAEAAEIDRLNIFHATLLAMQRAVSALNVTPDYVLIDGNRCPILPMPAMAIVKGDSRVAEISAASILAKVSRDREMAELHQAFPEYGFAQHKGYPTVYHLEKLALHGATVHHRRSFAPVKRVLGLL

SEQ ID NO: 16 - protein, 198 aa, Candidatus Sodalis sp. SoCistrobi
MTATFIYPAATLIAGVDEVGRGPLVGAVVTAAVILDPARPVLGLADSKKLSEKRREALYVEITRCALAWSVGRAEASEIDSINIYQATLLAMQRAVAGLAVVPDFVLVDGNRCPLLPMPSQAIVKGDSRVAEISAASIIAKVTRDREMAALHLQFPEYGFAQHKGYPTAFHLEKLALHGATVHHRRSFAPVRRVLELA

SEQ ID NO: 17 - protein, 197 aa, Providencia heimbachae
MDFIYPKANLIAGVDEVGRGPLVGAVVTAAVILDPNNPIVGLADSKKLTEKKREKLFDEIKEKALCWCIGRAEPEEIDKINILHATMLAMQRAVAGLSITPDFVLVDGNRCPELLMPSQAVVKGDSLVQEISAASILAKVVRDREMVELDKIFPEYGFAKHKGYPTPYHLEKLAQHGATEFHRKSFAPVRRALEIKQ

SEQ ID NO: 18 - protein, 208 aa, Erwiniaceae
MSEFIYPLANRIAGVDEVGRGPLVGAVVTAAVILDPARPIAGLADSKKLSEKRRLALYELITTHALSWSVGRAEPEEIDQLNILHATMLAMQRAVAGLSEVPDYVLIDGNRCPQLAMPALAVIKGDSLVAEISAASIIAKVTRDREMVELDRQYPEYGFAQHKGYPTALHREKLIKYGATPFHRRSFAPVRNALLDAEVMRDSASRTD

SEQ ID NO: 19 - protein, 196 aa, Proteus mirabilis
MEFVYPKANLIAGIDEVGRGPLVGAVVTAAVILDPANPIQGLMDSKKLTEKKRNALYDEIKEKALCWAIGRAEPEEIDKLNILWATMKAMERAVAGLSITPDMVLVDGNRCPNLPMASQAVIKGDSLVQEISAASILAKVTRDREMEQLDKLYPDYGFAKHKGYPTAFHMEKLASLGATPYHRKSFAPVKRALNLV

SEQ ID NO: 20 - protein, 195 aa, Haemophilus sputorum
MFIYPKAKLIAGVDEVGRGPLVGAVVTAAVILDPQKPIMGLTDSKKLSEKKRLALAEEIKEKARCWSLGRAEPEEIDSLNILHATMLAMQRAVEGLSITPDFVLVDGNRLPNLSMPAQAVVKGDALVQEISAASILAKVTRDLEMAELDKQFPEYGFAKHKGYPTALHFEKLSQYGATPFHRKSFAPVARCLNLK

SEQ ID NO: 21 - protein, 201 aa, Salinivibrio sp. HTSP
MTMTEHAFQYPDAQLIAGVDEVGRGPLVGAVVTAAVILDPAQPIVGLTDSKKLSEKKRLALYDEIKQKALAWSVGRAEPDEIDSLNILHATMLAMQRAVDGLSVMPDYALIDGNRVPPLSMPAEAVVKGDLRVAEISAASILAKVDRDHEMAMLDAAYPNYGFAQHKGYPTKVHMAALAEHGALPMHRKSFKPVKRALGID

SEQ ID NO: 22 - protein, 198 aa, Vibrio parahaemolyticus
MIEFVYPHTHLVAGVDEVGRGPLVGAVVTAAVILDPARPIVGLNDSKKLSEKRRLALYDEIKEKALSWSLGRAEPHEIDELNILHATMLAMQRAVAGLHIAPEYVLIDGNRCPALPVPSLAVVKGDSRVAEISAASILAKVTRDAEMAALDSVFPQYGFAQHKGYPTAFHLEKLAEHGATEHHRRSFAPVKRALGLAS

SEQ ID NO: 23 - protein, 198 aa, Leclercia adecarboxylata
MMEFIYPHTHLVAGVDEVGRGPLVGAVVTAAVILDPARPIIGLNDSKKLSEKRRLALYDEIKEKALAWSLGRAEPHEIDELNILHATMLAMQRAVAGLKVVPEYVLIDGNRCPALPMPSLAVVKGDSRVAEISAASIIAKVTRDAEMAALDITFPQYGFAQHKGYPTAFHLERLAEHGATEHHRRSFGPVKRALGLMS

SEQ ID NO: 24 - protein, 198 aa, Kluyvera intermedia
MMEFVYPHTHLVAGVDEVGRGPLVGAVVTAAVILDPARPIIGLNDSKKLSEKRRLALYDEIKEKALAWSLGRAEPHEIDELNILHATMLAMQRAVAGLGIIPEYVLIDGNRCPSLPMPSLAVVKGDSRVPEISAASILAKVTRDAEMATLDMTFPQYGFAQHKGYPTAFHLEKLAEHGATEHHRRSFAPVKRVLGLVS

SEQ ID NO: 25 - protein, 198 aa, Grimontella sp. AG753
MMEFIYPHTHLVAGVDEVGRGPLVGAVVTAAVILDPARPIIGLNDSKKLSEKRRLALFDEIKEKALAWSLGRAEPHEIDELNILHATMLAMQRAVAGLGIIPEYVLIDGNRCPKLPMPSLAVVKGDSRVPEISAASILAKVTRDAEMATLDLTFPQYGFAQHKGYPTAFHLEKLAEHGATEHHRRSFAPVKRVLGLVS

SEQ ID NO: 26 - protein, 198 aa, Kluyvera intestini; identical to SEQ ID NO: 25

SEQ ID NO: 27 - protein, 198 aa, Raoultella sp. 10-1
MIEFVYPHTHLVAGVDEVGRGPLVGAVVTAAVILDPAKPITGLNDSKKLSEKRRLALFAEIKEKALSWSLGRAEPHEIDELNILHATMLAMQRAVAGLHIAPEFVLIDGNRCPSLPVPSLAVVKGDSRVAEISAASILAKVTRDAEMVTLDLEFPQYGFAQHKGYPTAFHLEKLIEHGATEHHRRSFGPVKRALGLAS

SEQ ID NO: 28 - protein, 198 aa, Phytobacter ursingii
MMEFVYPHTHLVAGVDEVGRGPLVGAVVTAAVILDPARPIIGLNDSKKLSEKRRLSLYDEIKEKALAWSLGRAEPHEIDELNILHATMLAMQRAVAGLGIIPEYVLIDGNRCPSLPMPSLAVVKGDSRVPEISAASILAKVTRDAEMATLDMTFPQYGFAQHKGYPTAFHLEKLAEHGATEHHRRSFAPVKRVLGLVS

SEQ ID NO: 29 - protein, 198 aa, Kosakonia sacchari
MIEFVYPHTHLVAGVDEVGRGPLVGAVVTAAVILDPERPIVGLNDSKKLSEKRRLSLCDEIKEKALAWSLGRAEPHEIDELNILHATMLAMQRAVAGLAIAPEFVLIDGNRCPALPMPSLAVVKGDSRVAEISAASILAKVTRDAEMAALDIIFPQYGFAQHKGYPTAFHLERLAEHGATEHHRRSFAPVKRALGLAS

SEQ ID NO: 30 - protein, 198 aa, Metakosakonia massiliensis
MMEFIYPHTHLVAGVDEVGRGPLVGAVVTAAVILDPARPIVGLNDSKKLSEKRRLALYDEIKEKALAWSLGRAEPHEIDELNILHATMLAMQRAVAGLGITPEFVLIDGNRCPTLPMPSLAVVKGDSRVAEISAASILAKVTRDAEMATLDLSFPQYGFAQHKGYPTAFHLERLAEHGATEHHRRSFGPVKRALGLVS

SEQ ID NO: 31 - protein, 198 aa, Lelliottia nimipressuralis
MMEFVYPHTHLVAGVDEVGRGPLVGAVVTAAVILDPARPIVGLNDSKKLSEKRRLALFDEIKEKALAWSLGRAEPEEIDTLNILHATMLAMQRAVAGLNIVPEYVLIDGNRCPALPMPSMAVVKGDSRVAEISAASIIAKVTRDAEMAALDLTFPQYGFAQHKGYPTAFHLERLAEHGATEHHRRSFGPVKRALGLVS

SEQ ID NO: 32 - protein, 198 aa, Trabulsiella odontotermitis
MMEFIYPHTHLVAGVDEVGRGPLVGAVVTAAVILDPARPIVGLNDSKKLSEKRRLALFDEITEKALCWSLGRAEPHEIDELNILHATMLAMQRAVAGLKIAPEYVLIDGNRCPALPMPSMAVVKGDSRVQEISAASILAKVTRDAEMTALDLNFPQYGFAQHKGYPTAFHLEKLAEHGATEHHRRSFAPVKRALGLVS

SEQ ID NO: 33 - protein, 198 aa, Metakosakonia sp. MRY16-398
MMEFIYPHTHLVAGVDEVGRGPLVGAVVTAAVILDPARPIIGLNDSKKLSEKRRLALFDEIKEKALAWGLGRAEPHEIDELNILHATMLAMQRAVAGLGIIPEYVLIDGNRCPKLPMPSLAVVKGDSRVPEISAASILAKVTRDAEMATLDLTFPQYGFAQHKGYPTAFHLEKLAEHGATEHHRRSFAPVKRVLGLVS

SEQ ID NO: 34 - protein, 198 aa, Cedecea lapagei
MMEFIYPHTHLVAGVDEVGRGPLVGAVVTAAVILDPARPIVGLNDSKKLSEKRRLALFDEIKEKALAWSLGRAEPEEIDTLNILHATMLAMQRAVAGLNIVPEYVLIDGNRCPALPMPSMAVVKGDSRVAEISAASIIAKVTRDAEMAALDLTFPQYGFAQHKGYPTAFHLERLAEHGATEHHRRSFGPVKRALGLVS

SEQ ID NO: 35 - protein, 198 aa, Kosakonia sp. AG348
MIEFVYPHTHLVAGVDEVGRGPLVGAVVTAAVILDPKRPIIGLNDSKKLSEKRRLSLCDEIKEKALAWSLGRAEPHEIDELNILHATMLAMQRAVAGLAIAPEFVLIDGNRCPALPMPSLAVVKGDSRVAEISAASILAKVTRDAEMAELDIIFPQYGFAQHKGYPTAFHLERLAEHGATEHHRRSFAPVKRALGLAS

SEQ ID NO: 36 - protein, 198 aa, Franconibacter pulveris
MMEFIYPHTQLVAGVDEVGRGPLVGAVVTAAVILDPARPIIGLADSKKLSEKRRLALFDEIREKALAWSLGRAEPHEIDELNILHATMLAMQRAVAGLAIAPEYVLIDGNRCPKLPVPAMAVVKGDSRVAEISAASILAKVTRDAEMAELDLSFPQYGFAQHKGYPTAFHLERLAEHGATIHHRRSFAPVKRALGLAS

SEQ ID NO: 37 - protein, 198 aa, Trabulsiella guamensis
MMEFIYPHTHLVAGVDEVGRGPLVGAVVTAAVILDPARPITGLNDSKKLSEKRRLALFDEITEKALCWSLGRAEPHEIDELNILHATMLAMQRAVAGLTIAPEYVLIDGNRCPALSMPSMAVVKGDSRVQEISAASILAKVTRDAEMTALDLNFPQYGFAQHKGYPTAFHLEKLAEHGATEHHRRSFAPVKRALGLVS

SEQ ID NO: 38 - protein, 198 aa, Yokenella regensburgei
MIEFIYPHTHLVAGVDEVGRGPLVGAVVTAAVILDPAQPIVGLNDSKKLSEKRRLALFDEIKEKALSWSLGRAEPHEIDELNILHATMLAMQRAVAGLHIPPEYVLIDGNRCPALPVPSMAVVKGDSRVAEISAASILAKVTRDAEMAELDLTFPQYGFAQHKGYPTAFHLEKLALHGATEHHRRSFAPVKRVLGLVS

SEQ ID NO: 39 - protein, 198 aa, Mesorhizobium sp.
MMEFVYPHTHLVAGVDEVGRGPLVGAVVTAAVILDPARPIIGLNDSKKLSEKRRLALFSEIQEKALAWSLGRAEPHEIDELNILHATMLAMQRAVAGLKISPEYVLIDGNRCPALPMPSMAVVKGDSRVAEISAASIIAKVSRDAEMAELDLTYPQYGFAQHKGYPTAFHLERLAEHGATEHHRRSFGPVKRALGLVS

SEQ ID NO: 40 - protein, 198 aa, Atlantibacter subterranea
MIEFIYPHTQLVAGVDEVGRGPLVGAVVTAAVILDPSRPILGLADSKKLSEKRRLALFDEITEKALCWSLGRAEPHEIDELNILHATMLAMQRAVAGLSVTPEYVLIDGNRCPQLPMPSMAVVKGDSRVAEISAASILAKVTRDAEMAALDISFPQYGFAQHKGYPTAFHLERLAEHGATEHHRRSFAPVRRALNLVS

SEQ ID NO: 41 - protein, 198 aa, Cronobacter sakazakii
MMEFIYPHTHLVAGVDEVGRGPLVGAVVTAAVILDPARPIVGLNDSKKLSEKRRLALFDEIKEKALAWSLGRAEPEEIDDLNILHATMLAMQRAVAGLKIVPEYVLIDGNRCPALPMPSMAVVKGDSRVAEISAASIIAKVTRDAEMAALDLTYPAYGFAQHKGYPTAFHLEKLAEHGATEHHRRSFGPVKRALGLVS

SEQ ID NO: 42 - protein, 198 aa, Scandinavium goeteborgense
MTDIFIYPHTHLVAGVDEVGRGPLVGAVVTAAVILDPARPIIGLNDSKKLSEKRRLALFDEIKEKALSWSLGRAEPHEIDELNILHATMLAMQRAVAGLHISPEYVLIDGNRCPALPVPSLAVVKGDSRVAEISAASILAKVSRDAEMAALDITFPEYGFAQHKGYPTAFHLEKLALHGATEHHRRSFGPVKRALGIA

SEQ ID NO: 43 - DNA, 62 bp, synthetic construct
  misc_feature 1..62: note = Adaptor sequence
  misc_feature 47..54: note = n is a, t, g, or c
  source 1..62: mol_type = other DNA
gaatttaatacgactcactatagggtacacgacgctcttccgatctnnnnnnnngcttaacg

SEQ ID NO: 44 - DNA, 48 bp, synthetic construct
  misc_feature 1..48: note = Adaptor sequence
  misc_feature 10..17: note = n is a, t, c, or g
  misc_feature 40..48: note = the region contains exonuclease-resistant phosphothioate linkage
  source 1..48: mol_type = other DNA
cgttraagcnnnnnnnnagatcggaagagcgtcgtgtacccccccccc

SEQ ID NO: 45 - DNA, 62 bp, synthetic construct
  misc_feature 1..62: note = Adaptor sequence
  misc_feature 47..54: note = n is a, t, g, or c
  source 1..62: mol_type = other DNA
gaatttaatacgactcactatagggtacacgacgctcttccgatctnnnnnnnncgatccta

SEQ ID NO: 46 - DNA, 48 bp, synthetic construct
  misc_feature 1..48: note = Adaptor sequence
  misc_feature 10..17: note = n is a, t, g, or c
  misc_feature 40..48: note = the region contains exonuclease-resistant phosphothioate linkage
  source 1..48: mol_type = other DNA
taggratcgnnnnnnnnagatcggaagagcgtcgtgtacccccccccc

SEQ ID NO: 47 - DNA, 62 bp, synthetic construct
  misc_feature 1..62: note = Adaptor sequence
  misc_feature 47..54: note = n is a, t, g, or c
  source 1..62: mol_type = other DNA
gaatttaatacgactcactatagggtacacgacgctcttccgatctnnnnnnnngcaactac

SEQ ID NO: 48 - DNA, 48 bp, synthetic construct
  misc_feature 1..48: note = Adaptor sequence
  misc_feature 6: note = n is u
  misc_feature 10..17: note = n is a, t, g, or c
  misc_feature 40..48: note = the region contains exonuclease-resistant phosphothioate linkage
  source 1..48: mol_type = other DNA
gtagrntgcnnnnnnnnagatcggaagagcgtcgtgtacccccccccc

SEQ ID NO: 49 - DNA, 62 bp, synthetic construct
  misc_feature 1..62: note = Adaptor sequence
  misc_feature 47..54: note = n is a, t, g, or c
  source 1..62: mol_type = other DNA
gaatttaatacgactcactatagggtacacgacgctcttccgatctnnnnnnnngtactcct

SEQ ID NO: 50 - DNA, 48 bp, synthetic construct
  misc_feature 1..48: note = Adaptor sequence
  misc_feature 10..17: note = n is a, t, g, or c
  misc_feature 40..48: note = the region contains exonuclease-resistant phosphothioate linkage
  source 1..48: mol_type = other DNA
aggargtacnnnnnnnnagatcggaagagcgtcgtgtacccccccccc

SEQ ID NO: 51 - DNA, 62 bp, synthetic construct
  misc_feature 1..62: note = Adaptor sequence
  misc_feature 47..54: note = n is a, t, g, or c
  source 1..62: mol_type = other DNA
gaatttaatacgactcactatagggtacacgacgctcttccgatctnnnnnnnngactgttg

SEQ ID NO: 52 - DNA, 48 bp, synthetic construct
  misc_feature 1..48: note = Adaptor sequence
  misc_feature 10..17: note = n is a, t, g, or c
  misc_feature 40..48: note = the region contains exonuclease-resistant phosphothioate linkage
  source 1..48: mol_type = other DNA
caacragtcnnnnnnnnagatcggaagagcgtcgtgtacccccccccc

SEQ ID NO: 53 - DNA, 62 bp, synthetic construct
  misc_feature 1..62: note = Adaptor sequence
  misc_feature 47..54: note = n is a, t, g, or c
  source 1..62: mol_type = other DNA
gaatttaatacgactcactatagggtacacgacgctcttccgatctnnnnnnnnacaagcca

SEQ ID NO: 54 - DNA, 47 bp, synthetic construct
  misc_feature 1..47: note = Adaptor sequence
  misc_feature 5: note = n is u
  misc_feature 9: note = n is a, c, g, or t
  misc_feature 10..17: note = n is a, t, g, or c
  misc_feature 39..47: note = the region contains exonuclease-resistant phosphothioate linkage
  source 1..47: mol_type = other DNA
ggcrntgtnnnnnnnnagatcggaagagcgtcgtgtacccccccccc

SEQ ID NO: 55 - DNA, 62 bp, synthetic construct
  misc_feature 1..62: note = Adaptor sequence
  misc_feature 47..54: note = n is a, t, g, or c
  source 1..62: mol_type = other DNA
gaatttaatacgactcactatagggtacacgacgctcttccgatctnnnnnnnnatccgtac

SEQ ID NO: 56 - DNA, 48 bp, synthetic construct
  misc_feature 1..48: note = Adaptor sequence
  misc_feature 10..17: note = n is a, t, g, or c
  misc_feature 40..48: note = the region contains exonuclease-resistant phosphothioate linkage
  source 1..48: mol_type = other DNA
gtacrggatnnnnnnnnagatcggaagagcgtcgtgtacccccccccc

SEQ ID NO: 57 - DNA, 62 bp, synthetic construct
  misc_feature 1..62: note = Adaptor sequence
  misc_feature 47..54: note = n is a, t, g, or c
  source 1..62: mol_type = other DNA
gaatttaatacgactcactatagggtacacgacgctcttccgatctnnnnnnnncacagcat

SEQ ID NO: 58 - DNA, 48 bp, synthetic construct
  misc_feature 1..48: note = Adaptor sequence
  misc_feature 6: note = n is u
  misc_feature 10..17: note = n is a, t, g, or c
  misc_feature 40..48: note = the region contains exonuclease-resistant phosphothioate linkage
  source 1..48: mol_type = other DNA
atgcrngtgnnnnnnnnagatcggaagagcgtcgtgtacccccccccc

SEQ ID NO: 59 - DNA, 62 bp, synthetic construct
  misc_feature 1..62: note = Adaptor sequence
  misc_feature 47..54: note = n is a, t, g, or c
  source 1..62: mol_type = other DNA
gaatttaatacgactcactatagggtacacgacgctcttccgatctnnnnnnnnaagacgtg

SEQ ID NO: 60 - DNA, 48 bp, synthetic construct
  misc_feature 1..48: note = Adaptor sequence
  misc_feature 6: note = n is u
  misc_feature 10..17: note = n is a, t, g, or c
  misc_feature 40..48: note = the region contains exonuclease-resistant phosphothioate linkage
  source 1..48: mol_type = other DNA
cacgrncttnnnnnnnnagatcggaagagcgtcgtgtacccccccccc

SEQ ID NO: 61 - DNA, 62 bp, synthetic construct
  misc_feature 1..62: note = Adaptor sequence
  misc_feature 47..54: note = n is a, t, g, or c
  source 1..62: mol_type = other DNA
gaatttaatacgactcactatagggtacacgacgctcttccgatctnnnnnnnnccacaaga

SEQ ID NO: 62 - DNA, 48 bp, synthetic construct
  misc_feature 1..48: note = Adaptor sequence
  misc_feature 10..17: note = n is a, t, g, or c
  misc_feature 40..48: note = the region contains exonuclease-resistant phosphothioate linkage
  source 1..48: mol_type = other DNA
tcttrgtggnnnnnnnnagatcggaagagcgtcgtgtacccccccccc

SEQ ID NO: 63 - DNA, 62 bp, synthetic construct
  misc_feature 1..62: note = Adaptor sequence
  misc_feature 47..54: note = n is a, t, g, or c
  source 1..62: mol_type = other DNA
gaatttaatacgactcactatagggtacacgacgctcttccgatctnnnnnnnnagttctgc

SEQ ID NO: 64 - DNA, 48 bp, synthetic construct
  misc_feature 1..48: note = Adaptor sequence
  misc_feature 10..17: note = n is a, t, g, or c
  misc_feature 40..48: note = the region contains exonuclease-resistant phosphothioate linkage
  source 1..48: mol_type = other DNA
gcagraactnnnnnnnnagatcggaagagcgtcgtgtacccccccccc

SEQ ID NO: 65 - DNA, 62 bp, synthetic construct
  misc_feature 1..62: note = Adaptor sequence
  misc_feature 47..54: note = n is a, t, g, or c
  source 1..62: mol_type = other DNA
gaatttaatacgactcactatagggtacacgacgctcttccgatctnnnnnnnnctagcgat

SEQ ID NO: 66 - DNA, 48 bp, synthetic construct
  misc_feature 1..48: note = Adaptor sequence
  misc_feature 10..17: note = n is a, t, g, or c
  misc_feature 40..48: note = the region contains exonuclease-resistant phosphothioate linkage
  source 1..48: mol_type = other DNA
atcgrctagnnnnnnnnagatcggaagagcgtcgtgtacccccccccc

SEQ ID NO: 67 - DNA, 62 bp, synthetic construct
  misc_feature 1..62: note = Adaptor sequence
  misc_feature 47..54: note = n is a, t, g, or c
  source 1..62: mol_type = other DNA
gaatttaatacgactcactatagggtacacgacgctcttccgatctnnnnnnnntacgcaag

SEQ ID NO: 68 - DNA, 48 bp, synthetic construct
  misc_feature 1..48: note = Adaptor sequence
  misc_feature 10..17: note = n is a, t, g, or c
  misc_feature 40..48: note = the region contains exonuclease-resistant phosphothioate linkage
  source 1..48: mol_type = other DNA
cttgrcgtannnnnnnnagatcggaagagcgtcgtgtacccccccccc

SEQ ID NO: 69 - DNA, 62 bp, synthetic construct
  misc_feature 1..62: note = Adaptor sequence
  misc_feature 47..54: note = n is a, t, g, or c
  source 1..62: mol_type = other DNA
gaatttaatacgactcactatagggtacacgacgctcttccgatctnnnnnnnnctcactca

SEQ ID NO: 70 - DNA, 48 bp, synthetic construct
  misc_feature 1..48: note = Adaptor sequence
  misc_feature 6: note = n is u
  misc_feature 10..17: note = n is a, t, g, or c
  misc_feature 40..48: note = the region contains exonuclease-resistant phosphothioate linkage
  source 1..48: mol_type = other DNA
tgagrngagnnnnnnnnagatcggaagagcgtcgtgtacccccccccc

SEQ ID NO: 71 - DNA, 62 bp, synthetic construct
  misc_feature 1..62: note = Adaptor sequence
  misc_feature 47..54: note = n is a, t, g, or c
  source 1..62: mol_type = other DNA
gaatttaatacgactcactatagggtacacgacgctcttccgatctnnnnnnnntaaggctc

SEQ ID NO: 72 - DNA, 48 bp, synthetic construct
  misc_feature 1..48: note = Adaptor sequence
  misc_feature 10..17: note = n is a, t, g, or c
  misc_feature 40..48: note = the region contains exonuclease-resistant phosphothioate linkage
  source 1..48: mol_type = other DNA
gagcrcttannnnnnnnagatcggaagagcgtcgtgtacccccccccc

SEQ ID NO: 73 - DNA, 62 bp, synthetic construct
  misc_feature 1..62: note = Adaptor sequence
  misc_feature 47..54: note = n is a, t, g, or c
  source 1..62: mol_type = other DNA
gaatttaatacgactcactatagggtacacgacgctcttccgatctnnnnnnnnggtccaat

SEQ ID NO: 74 - DNA, 48 bp, synthetic construct
  misc_feature 1..48: note = Adaptor sequence
  misc_feature 10..17: note = n is a, t, g, or c
  misc_feature 40..48: note = the region contains exonuclease-resistant phosphothioate linkage
  source 1..48: mol_type = other DNA
attgrgaccnnnnnnnnagatcggaagagcgtcgtgtacccccccccc

SEQ ID NO: 75 - DNA, 62 bp, synthetic construct
  misc_feature 1..62: note = Adaptor sequence
  misc_feature 47..54: note = n is a, t, g, or c
  source 1..62: mol_type = other DNA
gaatttaatacgactcactatagggtacacgacgctcttccgatctnnnnnnnntagtacgg

SEQ ID NO: 76 - DNA, 48 bp, synthetic construct
  misc_feature 1..48: note = Adaptor sequence
  misc_feature 10..17: note = n is a, t, g, or c
  misc_feature 40..48: note = the region contains exonuclease-resistant phosphothioate linkage
  source 1..48: mol_type = other DNA
ccgtractannnnnnnnagatcggaagagcgtcgtgtacccccccccc

SEQ ID NO: 77 - DNA, 62 bp, synthetic construct
  misc_feature 1..62: note = Adaptor sequence
  misc_feature 47..54: note = n is a, t, g, or c
  source 1..62: mol_type = other DNA
gaatttaatacgactcactatagggtacacgacgctcttccgatctnnnnnnnnagtctgca

SEQ ID NO: 78 - DNA, 48 bp, synthetic construct
  misc_feature 1..48: note = Adaptor sequence
  misc_feature 10..17: note = n is a, t, g, or c
  misc_feature 40..48: note = the region contains exonuclease-resistant phosphothioate linkage
  source 1..48: mol_type = other DNA
tgcargactnnnnnnnnagatcggaagagcgtcgtgtacccccccccc

SEQ ID NO: 79 - DNA, 62 bp, synthetic construct
  misc_feature 1..62: note = Adaptor sequence
  misc_feature 47..54: note = n is a, t, g, or c
  source 1..62: mol_type = other DNA
gaatttaatacgactcactatagggtacacgacgctcttccgatctnnnnnnnnttgcaacc

SEQ ID NO: 80 - DNA, 48 bp, synthetic construct
  misc_feature 1..48: note = Adaptor sequence
  misc_feature 10..17: note = n is a, t, g, or c
  misc_feature 40..48: note = the region contains exonuclease-resistant phosphothioate linkage
  source 1..48: mol_type = other DNA
ggttrgcaannnnnnnnagatcggaagagcgtcgtgtacccccccccc

SEQ ID NO: 81 - DNA, 62 bp, synthetic construct
  misc_feature 1..62: note = Adaptor sequence
  misc_feature 47..54: note = n is a, t, g, or c
  source 1..62: mol_type = other DNA
gaatttaatacgactcactatagggtacacgacgctcttccgatctnnnnnnnncagcttgt

SEQ ID NO: 82 - DNA, 48 bp, synthetic construct
  misc_feature 1..48: note = Adaptor sequence
  misc_feature 10..17: note = n is a, t, g, or c
  misc_feature 40..48: note = the region contains exonuclease-resistant phosphothioate linkage
  source 1..48: mol_type = other DNA
acaargctgnnnnnnnnagatcggaagagcgtcgtgtacccccccccc

SEQ ID NO: 83 - DNA, 62 bp, synthetic construct
  misc_feature 1..62: note = Adaptor sequence
  misc_feature 47..54: note = n is a, t, g, or c
  source 1..62: mol_type = other DNA
gaatttaatacgactcactatagggtacacgacgctcttccgatctnnnnnnnnagacacag

SEQ ID NO: 84 - DNA, 48 bp, synthetic construct
  misc_feature 1..48: note = Adaptor sequence
  misc_feature 10..17: note = n is a, t, g, or c
  misc_feature 40..48: note = the region contains exonuclease-resistant phosphothioate linkage
  source 1..48: mol_type = other DNA
ctgtrgtctnnnnnnnnagatcggaagagcgtcgtgtacccccccccc

SEQ ID NO: 85 - DNA, 62 bp, synthetic construct
  misc_feature 1..62: note = Adaptor sequence
  misc_feature 47..54: note = n is a, t, g, or c
  source 1..62: mol_type = other DNA
gaatttaatacgactcactatagggtacacgacgctcttccgatctnnnnnnnnatggcaga

SEQ ID NO: 86 - DNA, 48 bp, synthetic construct
  misc_feature 1..48: note = Adaptor sequence
  misc_feature 10..17: note = n is a, t, g, or c
  misc_feature 40..48: note = the region contains exonuclease-resistant phosphothioate linkage
  source 1..48: mol_type = other DNA
tctgrccatnnnnnnnnagatcggaagagcgtcgtgtacccccccccc

SEQ ID NO: 87 - DNA, 62 bp, synthetic construct
  misc_feature 1..62: note = Adaptor sequence
  misc_feature 47..54: note = n is a, t, g, or c
  source 1..62: mol_type = other DNA
gaatttaatacgactcactatagggtacacgacgctcttccgatctnnnnnnnngacatacc

SEQ ID NO: 88 - DNA, 48 bp, synthetic construct
  misc_feature 1..48: note = Adaptor sequence
  misc_feature 6: note = n is u
  misc_feature 10..17: note = n is a, t, g, or c
  misc_feature 40..48: note = the region contains exonuclease-resistant phosphothioate linkage
  source 1..48: mol_type = other DNA
ggtarngtcnnnnnnnnagatcggaagagcgtcgtgtacccccccccc

SEQ ID NO: 89 - DNA, 62 bp, synthetic construct
  misc_feature 1..62: note = Adaptor sequence
  misc_feature 47..54: note = n is a, t, g, or c
  source 1..62: mol_type = other DNA
gaatttaatacgactcactatagggtacacgacgctcttccgatctnnnnnnnngcgttgtt

SEQ ID NO: 90 - DNA, 48 bp, synthetic construct
  misc_feature 1..48: note = Adaptor sequence
  misc_feature 10..17: note = n is a, t, g, or c
  misc_feature 40..48: note = the region contains exonuclease-resistant phosphothioate linkage
  source 1..48: mol_type = other DNA
aacaracgcnnnnnnnnagatcggaagagcgtcgtgtacccccccccc

SEQ ID NO: 91 - DNA, 68 bp, synthetic construct
  misc_feature 1..68: note = Adaptor sequence
  misc_feature 47..54: note = n is a, t, g, or c
  misc_feature 55..59: note = n is a, c, g, or t
  source 1..68: mol_type = other DNA
cccccgaatttaatacgactcactatagggtacacgacgctcttccgatctnnnnnnnnctaccaggg

SEQ ID NO: 92 - DNA, 70 bp, synthetic construct
  misc_feature 1..70: note = Adaptor sequence
  misc_feature 10..17: note = n is a, t, g, or c
  misc_feature 63..70: note = the region contains exonuclease-resistant phosphothioate linkage
  source 1..70: mol_type = other DNA
ccctggtagnnnnnnnnagatcggaagagcgtcgtgtaccctatagtgagtcgtattaaattcccccccc

SEQ ID NO: 93 - DNA, 63 bp, synthetic construct
  misc_feature 1..63: note = Adaptor sequence
  misc_feature 47..54: note = n is a, t, g, or c
  source 1..63: mol_type = other DNA
gaatttaatacgactcactatagggtacacgacgctcttccgatctnnnnnnnnctaccaggg

SEQ ID NO: 94 - DNA, 49 bp, synthetic construct
  misc_feature 1..49: note = Adaptor sequence
  misc_feature 11..18: note = n is a, t, g, or c
  misc_feature 40..49: note = the region contains exonuclease-resistant phosphothioate linkage
  source 1..49: mol_type = other DNA
crcctggtagnnnnnnnnagatcggaagagcgtcgtgtacccccccccc

SEQ ID NO: 95 - DNA, 49 bp, synthetic construct
  misc_feature 1..49: note = Adaptor sequence
  misc_feature 11..18: note = n is a, t, g, or c
  misc_feature 40..49: note = the region contains exonuclease-resistant phosphothioate linkage
  source 1..49: mol_type = other DNA
ccctrggtagnnnnnnnnagatcggaagagcgtcgtgtacccccccccc

SEQ ID NO: 96 - DNA, 62 bp, synthetic construct
  misc_feature 1..62: note = Adaptor sequence
  misc_feature 47..54: note = n is a, t, g, or c
  source 1..62: mol_type = other DNA
gaatttaatacgactcactatagggtacacgacgctcttccgatctnnnnnnnnctaccagg

SEQ ID NO: 97 - DNA, 48 bp, synthetic construct
  misc_feature 1..48: note = Adaptor sequence
  misc_feature 10..17: note = n is a, t, g, or c
  misc_feature 40..48: note = the region contains exonuclease-resistant phosphothioate linkage
  source 1..48: mol_type = other DNA
cctggtargnnnnnnnnagatcggaagagcgtcgtgtacccccccccc

SEQ ID NO: 98 - DNA, 65 bp, synthetic construct
  misc_feature 1..65: note = Adaptor sequence
  misc_feature 47..54: note = n is a, t, g, or c
  source 1..65: mol_type = other DNA
gaatttaatacgactcactatagggtacacgacgctcttccgatctnnnnnnnnagcaattcaag

SEQ ID NO: 99 - DNA, 51 bp, synthetic construct
  misc_feature 1..51: note = Adaptor sequence
  misc_feature 12: note = n is u
  misc_feature 13..20: note = n is a, t, g, or c
  misc_feature 41..51: note = the region contains exonuclease-resistant phosphothioate linkage
  source 1..51: mol_type = other DNA
cttgaattgcrnnnnnnnnnagatcggaagagcgtcgtgtacccccccccc

SEQ ID NO: 100 - DNA, 67 bp, synthetic construct
  misc_feature 1..67: note = Adaptor sequence
  misc_feature 47..54: note = n is a, t, g, or c
  source 1..67: mol_type = other DNA
gaatttaatacgactcactatagggtacacgacgctcttccgatctnnnnnnnngtataacagaaac

SEQ ID NO: 101 - DNA, 53 bp, synthetic construct
  misc_feature 1..53: note = Adaptor sequence
  misc_feature 15..22: note = n is a, t, g, or c
  misc_feature 43..53: note = the region contains exonuclease-resistant phosphothioate linkage
  source 1..53: mol_type = other DNA
gtttctgttatarcnnnnnnnnagatcggaagagcgtcgtgtacccccccccc

SEQ ID NO: 102 - DNA, 25 bp, synthetic construct
  misc_feature 1..25: note = T7 promoter
  misc_feature 1..25: note = T7 promoter
  source 1..25: mol_type = other DNA
gaatttaatacgactcactataggg

SEQ ID NO: 103 - protein, 224 aa, Pyrococcus abyssi
MKVAGADEAGRGPVIGPLVIVAAVVEEDKIRSLTKLGVKDSKQLTPAQREKLFDEIVKVLDDYSVVIVSPQDIDGRKGSMNELEVENFVKALNSLKVKPEVIYIDSADVKAERFAENIRSRLAYEAKVVAEHKADAKYEIVSAASILAKVIRDREIEKLKAEYGDFGSGYPSDPRTKKWLEEWYSKHGNFPPIVRRTWDTAKKIEEKFKRAQLTLDNFLKRFRN

SEQ ID NO: 104 - protein, 222 aa, Pyrococcus sp. ST04
MKVGGIDEAGRGPAIGPLVIVAVVVDESKLSSLKNIGVKDSKQLTPEQRRRMFSEIVSLLEDYVVIKVPPSEIDNRSGTMNELEVEKFAEALNSLKVKPEVIYADAADVKAERFAREIGARLSYNASIIAEHKADAKYEVVSAASILAKVIRDEEIEKLKEEYGDFGSGYPSDPRTKKWLEEWFKKHKSFPPIVRRSWETVKKIEEKYKAQQLTLDSFFKKS

SEQ ID NO: 105 - protein, 221 aa, Pyrococcus yayanosii
MKVAGIDEAGRGPVLGPLVIVAVVVDEKKMTELEGIGVRDSKALTPKKREKLFERILSMVDDYSIVLVEPPEIDARAGTMNELEVEKFAQALNSLKVKPDVVYVDSADVRSERFGLALREKLAFDAKVVSEHKADAKYPVVSAASILAKVIRDREIEKLKLEYGDFGSGYPSDPRTRAFLEDYYRRHGDFPPMVRRTWKTVKEIEKQLGRKGQLTLDQFLP

SEQ ID NO: 106 - protein, 225 aa, Thermococcus paralvinellae
MKLGGIDEAGRGPVIGPLVIAAVVVDEKNLSKLEALGVKDSKKLTPERREKLFNEIIALLDDYVIIELSPEQIDERKGTMNEFEVENFIKALNSLKVKPDVLYIDAADVKEERFGEIIGKRLNFSPKIIAEHKADAKYLPVSAASILAKVTRDRAIEKLKEQYGEIGSGYPSDPRTRKFLEDYYKEHGEFPPIVRRSWKTLKKIEENLKARTQKKGQLNLLEFLK

SEQ ID NO: 107 - protein, 227 aa, Thermococcus sp. CX2
MKLAGIDEAGRGPVLGPMVIAAVVVDEKNVPKLEELGVRDSKKLTPKRRERLFDEIIRLLDDYVIVELWPEQIDSREGTLNEFEVDNFVKALNSLKVKPDVVYIDAADVKEARFGDEIGKRLDFKAEIIAEHKADDKFVPVSAASILAKVTRDRAIERLKEEYGEIGSGYPSDPRTRKFLEEYYRQHGDFPPIVRRSWKTLRKIEEKLSAEKKKRGQLTLGEFLRKG

SEQ ID NO: 108 - protein, 230 aa, Thermococcus barossii
MKLAGIDEAGRGPVIGPMVIAAIVVDEKNVPKLEELGVRDSKRLTPRRREKLFDEIIAVLDDYVILELLPEEIDSREGTLNEFEVENFVKALNSLKVKPDVVYIDAADVKEARFGEEVGKRLNFEAEIVAEHKADDKFVPVSAASILAKVTRDRAIEKLKEEYGEIGSGYPSDPRTRAFLESYYREHGDFPPIVRRGWKTLRKIEEKLRADVEAKKSRGRGQLSLDRFME

SEQ ID NO: 109 - protein, 226 aa, Thermococcus guaymasensis
MGKKLAGIDEAGRGPVIGPMVIAAVVVDEENVTNLEALGVKDSKKLTPRRRERLFDEIIEQLDDYAIVELWPEEIDSRDVSLNELEVENFARALNSLKVKPDIVYIDAADVKEGRFGEAIAKLLKFKAEIVAEHRADDKFIPVSAASILAKVRRDRAIEKLREEYGEIGSGYPSDPRTRDFLEKYYLEHGDFPPIVRRTWKTVEKIRKKLEERKRKPQLTLDSFLD

SEQ ID NO: 110 - protein, 233 aa, Thermococcus celer
MKLAGIDEAGRGPVIGPMVIAAVVLDEKNVPKLRDLGVRDSKKLTPKRRERLFNDIIKLLDDYVILELWPEEIDSRGGTLNELEVERFVEALNSLKVKPDVVYIDAADVKEGRFGEEIKERLNFEAKIVSEHRADDKFLPVSSASILAKVTRDRAIEKLKEKYGEIGSGYPSDPRTREFLENYYRQHGEFPPVVRRSWKTLRKIEEKLRKEAGSKNPENSKEKGQTSLDVFLR

SEQ ID NO: 111 - protein, 224 aa, Thermococcus zilligii
MGKKIAGIDEAGRGPVIGPMVIAAVVFDEDSIPNLKALGVRDSKKLTPRRREKLFDEILGIADDYVILELSPEEIDSREGTLNEFEVNNFAKALNSLKVKPDVIYIDAADVREERFGEEIGKFLNFKAEIIAEHKADDKFPPVSAASILAKVTRDRAIERLREEYGEIGSGYPSDPRTREFLMGYYKKHGEFPPVVRRTWETLKKIKVAEQPSIEEFLKGKRKN

SEQ ID NO: 112 - protein, 231 aa, Thermococcus sp. P6
MKLAGIDEAGRGPVIGPMVVAAVVVDEEKTEELRKLGVRDSKKLTPKRRAALFDEIIKVLDDYVILELSPEEIDSRGGTLNEFEVENFARALNSLGVKPDVVYVDAADVKEARFGADIEPRLNFKARIVSEHGADDRFIPVSAASILAKVTRDRAIERLREEYGEIGSGYPSDPRTREFLREYYVKHGEFPPIVRRSWKTLRKIEGEIKGRKSSRKQYGLDRFIGGSSPQP

SEQ ID NO: 113 - protein, 229 aa, Palaeococcus pacificus
MKLGGIDEAGRGPVIGPLVIATVVVDEKNLDRLRELNVRDSKKISPKRREELFNKIIEILDDYVVIELWPEEIDNRNGTLNEFEVENFIKALNSLKIKPEVLYIDAADVKEERFGEVIKKKLDFSPKIVSEHKADDKYLPVSAASILAKVTRDRAIEKLKEEYGEIGSGYPSDPRTRKFLEEYYLKYGDFPPIARRTWKTLKKLEEKLKPKLQKSSKKDGQLNITEFLR

SEQ ID NO: 114 - protein, 212 aa, Thermococci archaeon
EAGRGPVIGPMVVAAVVIEEGRVEDLSSIGVRDSKKLSPARRERLFEEILSTVDEIKVRVVPPEVVGDPAVNVNDLEVQVFGDVLNSLSLRPSVIYVDAADVDAERFASRLRERLSYEALIVAEHRADDRYPVVSAASIVAKVIRDREIEKIREVYGDVGSGYPSDPRTRRFLEDYLREHGDFPPVVRRSWKTLKKIREKSGRVTLDRFLGH

SEQ ID NO: 115 - protein, 224 aa, Crenarchaeota archaeon
MSSIVCGVDEAGRGPVIGPMVIAVACIEEENVGKLSEIGVKDSKELSRAQRQILYEKLRRILIFHDYVIVSPEEIDKYVRENKLNILELEKIKELVKKVLERFPDKRIIIYVDSPDVKAERFEKMLKNSLSSDRVEIYARHRADATIPIVSAASIIAKYVRDREIEKLKLRYGDFGSGYPSDPRTIRFLISYISRHGEPPPIARKTWRTCKNIIRELKKGKLFE

SEQ ID NO: 116 - protein, 220 aa, Euryarchaeota archaeon
MIAGIDEAGKGPVLGPMCVAGLMVDENKLDNILRLGVKDSKKLTPKKREALSVEIKKFADKIFILEVSPAQIDGLRKVMTMNEIMVACYVKVLEELKPESAFVDAADVIAERFGENIKKKYSRDLKITSEHKADEKYPIVSAASILAKVRRDELVRNLERTVGKEIGSGYPADPKTITFLESWVKEHGKLPDFARSSWETSKNIIEKFRKNQRTISDFFR

SEQ ID NO: 117 - protein, 216 aa, Candidatus Bathyarchaeota archaeon
MLAVGVDDAGRGSIIGPLVLAGVLHPEDKMEELKELGVKDSKRLTPTRRAKLAELIKSSVKAYHVVEIPPSEIDEKVGSGVKFRRLNFLEAKAAAEIIARLRPRVAYLDSCDVDAGRFAWQVSSLLPFKVKIVSEHGADAKYPIVAAASILAKVHRDQVIARLREAYGDFGSGYPSDPKTRSFLESWFKAHGSYPAFVRRTWKTLRRIPGRAGLNV

SEQ ID NO: 118 - protein, 222 aa, Thermoprotei archaeon
MRLGGVDDAGRGPIIGPLVIAGVCVDEGAMSSLQELGVRDSKTLSPSQREFLSREIRRLALKVCIAKVEPDEIDKYVGRTSMGKLNALEAKVMARIVEELGADVVYIDSPDINPDRYKRRILSFMSHTSKVKLVVENHADARYVIVAAASIIAKVERDRVIEQLKATYGDFGSGYPSDPRTVDFLTRWYEEHGDFPPIVRRSWATLDRIRRMVDMKKTRRLL

SEQ ID NO: 119 - protein, 219 aa, Candidatus Freyarchaeota archaeon
MFIAGVDEAGRGPVLGPIVCAGVLVREEDIPELVKLGVRDSKLLQPSKREALALDILKYAVKVAVKIMYPEEIDAARTNGLNLNELEAQIFAEIINQLKPDVTYVDAADVKPERFSQMIKNSLVVDTKLVSQHKADYKIPVVSAASIIAKVERDKEIRELKKFGDVGSGYCHDPKTISFLREWAREHGELPSFVRHSWITAKNILDELKQKVLDDFKSK

SEQ ID NO: 120 - protein, 228 aa, Candidatus Thorarchaeota archaeon
MSPSDSKLRGIAGIDEAGRGPLIGPLVVCGALFEQETIHDLNDLRVKDSKMLTPRRRTQLLEPIKRLASKIELLSISASEIDRLRGQKVNLNEIEVRAFVSVAQALKPSLLYLDAADVKAQRFGMAVSQRSGLSKLGCKVVSEHKADSKYPVVSAASIVAKVERDKAIKLLHEEYGDFGSGYPSDPKTIKFVRDILSESGELPNIVRHSWESVNRIRAELRTEQLRLG

SEQ ID NO: 121 - protein, 213 aa, Frankliniella occidentalis
MQIIKLHKQYWDLLMADFIYPVAHCIAGVDEVGRGPLVGAVVTAAVILDPNNPILGLADSKKISEKKRLMLCSEIKEKALSWSIGRAEPHEIDQLNILHATMLAMQRAVAGLSLTPDFVLIDGNRCPVLPMPAQAVVKGDSLVAEISAASILAKVTRDQEMADLDQQYPEYGFAQHKGYPTAKHLEQLIRFGPIPEHRRSFAPVRNILATLST

SEQ ID NO: 122 - protein, 501 aa, Oryza sativa Indica Group
MQAEGCEAWYEMEELAVMGVVEVLERLPRLLKIRKDLTRRFGELRPDVFVGIDAPDFNITLEGRLKQRGIRTIHYVSPSVWAWRQKRVFKIGKATDLVLAFLPFEKAFYDRFNVPCRFIGHTMADAMPLQPDRLAARAQLGIAPQARCLALLPGSRGAEVEMLSADFLKTAQLLRTRYPELEVVVPLVNAKRREQFERIKAEVAPDLTVHLLNGQGREAMIASDAALLASGTAALECMLAKCPMVVGYRMKPFTFWLAQKLVKTPYVSLPNLLAGREIVTELLQHDCVPDKLAAAVMPLLEESPETDALKQTFLTLHQSICCVGRGPLVGAVVTAAVILDPAQPIVGLADSKKLSEKRRLALYDEIVAKALSWSLGRAEPAEIDQLNILHATMLAMQRAVAGLHIAPDMVLIDGNRCPSLPMRSQAVVKGDSRVAEISAASILAKVTRDREMAELDSEFPDYGFAQHKGYPTAFHLERLAALGATEHHRRSFAPVKRALAL

SEQ ID NO: 123 - protein, 876 aa, Geobacillus stearothermophilus
MKNKLVLIDGNSVAYRAFFALPLLHNDKGIHTNAVYGFTMMLNKILAEEQPTHILVAFDAGKTTFRHETFQDYKGGRQQTPPELSEQFPLLRELLKAYRIPAYELDHYEADDIIGTMAARAEREGFAVKVISGDRDLTQLASPQVTVEITKKGITDIESYTPETVVEKYGLTPEQIVDLKGLMGDKSDNIPGVPGIGEKTAVKLLKQFGTVENVLASIDEIKGEKLKENLRQYRDLALLSKQLAAICRDAPVELTLDDIVYKGEDREKVVALFQELGFQSFLDKMAVQTDEGEKPLAGMDFAIADSVTDEMLADKAALVVEVVGDNYHHAPIVGIALANERGRFFLRPETALADPKFLAWLGDETKKKTMFDSKRAAVALKWKGIELRGVVFDLLLAAYLLDPAQAAGDVAAVAKMHQYEAVRSDEAVYGKGAKRTVPDEPTLAEHLVRKAAAIWALEEPLMDELRRNEQDRLLTELEQPLAGILANMEFTGVKVDTKRLEQMGAELTEQLQAVERRIYELAGQEFNINSPKQLGTVLFDKLQLPVLKKTKTGYSTSADVLEKLAPHHEIVEHILHYRQLGKLQSTYIEGLLKVVHPVTGKVHTMFNQALTQTGRLSSVEPNLQNIPIRLEEGRKIRQAFVPSEPDWLIFAADYSQIELRVLAHIAEDDNLIEAFRRGLDIHTKTAMDIFHVSEEDVTANMRRQAKAVNFGIVYGISDYGLAQNLNITRKEAAEFIERYFASFPGVKQYMDNIVQEAKQKGYVTTLLHRRRYLPDITSRNFNVRSFAERTAMNTPIQGSAADIIKKAMIDLSVRLREERLQARLLLQVHDELILEAPKEEIERLCRLVPEVMEQAVTLRVPLKVDYHYGPTWYDAK

SEQ ID NO: 124 - protein, 587 aa, Geobacillus stearothermophilus
DEGEKPLAGMDFAIADSVTDEMLADKAALVVEVVGDNYHHAPIVGIALANERGRFFLRPETALADPKFLAWLGDETKKKTMFDSKRAAVALKWKGIELRGVVFDLLLAAYLLDPAQAAGDVAAVAKMHQYEAVRSDEAVYGKGAKRTVPDEPTLAEHLVRKAAAIWALEEPLMDELRRNEQDRLLTELEQPLAGILANMEFTGVKVDTKRLEQMGAELTEQLQAVERRIYELAGQEFNINSPKQLGTVLFDKLQLPVLKKTKTGYSTSADVLEKLAPHHEIVEHILHYRQLGKLQSTYIEGLLKVVHPVTGKVHTMFNQALTQTGRLSSVEPNLQNIPIRLEEGRKIRQAFVPSEPDWLIFAADYSQIELRVLAHIAEDDNLIEAFRRGLDIHTKTAMDIFHVSEEDVTANMRRQAKAVNFGIVYGISDYGLAQNLNITRKEAAEFIERYFASFPGVKQYMDNIVQEAKQKGYVTTLLHRRRYLPDITSRNFNVRSFAERTAMNTPIQGSAADIIKKAMIDLSVRLREERLQARLLLQVHDELILEAPKEEIERLCRLVPEVMEQAVTLRVPLKVDYHYGPTWYDAK

SEQ ID NO: 125 - protein, 575 aa, Bacillus phage phi29 [sequence omitted]

SEQ ID NO: 126 - protein, 832 aa, unidentified [sequence omitted]